European Patent Application EP 4 276 114 A2, published November 15, 2023. Title: CD20 BINDING AGENTS. Applicant: VIB VZW. The sequence listing filed with the application follows.

SEQUENCE LISTING (169 sequences)

SEQ ID NO: 1 - DNA, 423 bp, Homo sapiens
  source 1..423: mol_type = unassigned DNA
caggtgcagctgcaggagtctgggggaggattggtgcaggctgggggctctctgagactctcctgtgcagcctctggacgcaccttcagtagacagtccatgggctggttccgccaggctccagggaaggagcgtgagtttgtagcagtcattacctggagtggtggcagcccatattatgcagactccgtgaggggccgattcaccatctccagagacaacgccaagaacaccgtgtatctgcaaatgaacagcctgaaacctgaggatacggccgtttattactgtgcagcccccgtttcgtacggtagtcagtggcttgcggactactggggccaggggacccaggtcaccgtctcctcagcggccgcatacccgtacgacgttccggactacggttcccaccaccatcaccatcactag

SEQ ID NO: 2 - DNA, 423 bp, Homo sapiens
  source 1..423: mol_type = unassigned DNA
caggtgcagctgcaggagtctgggggaggattggtgcaggctggggactctctgagactctcctgtgcagcctctggacgcaccttcagtagacagtccatgggctggttccgccaggctccagggaaggagcgtgagtttgtagcagtcattacctggagtggtggcagcccatattatgcagactccgtgaagggccgattcaccatctccagagacaacgccaagaacaccgtgtatctgcaaatgaacagcctgaaacctgaggatacggccgtttattactgtgcagcccccgtttcgtacggtagtcagtggcttgcggactactggggccaggggacccaggtcaccgtctcctcagcggccgcatacccgtacgacgttccggactacggttcccaccaccatcaccatcactag

SEQ ID NO: 3 - DNA, 423 bp, Homo sapiens
  source 1..423: mol_type = unassigned DNA
caggtgcagctgcaggagtctgggggaggattggtgcaggctgggggctctctgagactctcctgtgcagcctctggacgcaccttcagtagctatgccatgggctggttccgccaggctccagggaaggagcgtgagtttgtagcagtcattacctggagtggtggcagcccatattatgcagactccgtgaggggccgattcaccatctccagagacaacgccaagaacaccgtgtatctgcaaatgaacagcctgaaacctgaggatacggccgtttattactgtgcagcccccgtttcgtacggtagtcagtggcttgcggactactggggccaggggacccaggtcaccgtctcctcagcggccgcatacccgtacgacgttccggactacggttcccaccaccatcaccatcactag

SEQ ID NO: 4 - DNA, 423 bp, Homo sapiens
  source 1..423: mol_type = unassigned DNA
caggtgcagctgcaggagtctgggggaggattggtgcaagctgggggctctctgagactctcctgtgcagcctctggacgcaccttcagtagacagtccatgggctggttccgccaggctccaggggaggagcgtgagtttgtagcagtcattacctggagtggtggcagcccatattatgcagactccgtgaggggccgattcaccatctccagagacaacgccaagaacaccgtgtatctgcaaatgaacagcctgaaacctgaggatacggccgtttattactgtgcagcccccgtttcgtacggkagtcagtggcttgcggactactggggccaggggacccaggtcaccgtctcctcagcggccgcatacccgtacgacgttccggactacggttcccaccaccatcaccatcactag

SEQ ID NO: 5 - DNA, 423 bp, Homo sapiens
  source 1..423: mol_type = unassigned DNA
caggtgcagctgcaggagtctggaggaggattggtgcaggctgggggctctctgagactctcctgtgcagcctctggacgcaccttcagtggacagtccatgggctggttccgccaggctccagggaaggagcgtgagtttgtagcagtcattacctggagtggtggcagcccatattatgcagactccgtgaggggccgattcaccatctccagagacaacgccaagaacaccgtgcatctgcaaatgaacagcctgaaacctgaggatacggccgtttattactgtgcagcccccgtttcgtacggtagtcagtggcttgcggactactggggccaggggacccaggtcaccgtctcctcagcggccgcatacccgtacgacgttccggactacggttcccaccaccatcaccatcactag

SEQ ID NO: 6 - DNA, 423 bp, Homo sapiens
  source 1..423: mol_type = unassigned DNA
caggtgcagctgcaggagtctgggggaggattggtgcaggctgggggctctctgagactctcctgtgcagcctctggacgcaccttcagtagctataacatgggctggttccgccaggctccagggaaggagcgtgagtttgtagcagttattagctggagtggtggtagcccatactatgcggactccgtgaagggccgattcaccatctccagagacaacgccaagaacacggtgtatctgcaaatgaacagcctgaaacctgaggacacggccgtttattactgtgcagcccccgtttcgtacggtagtagctggcttgcggactactggggccaggggacccaggtcaccgtctcctcagcggccgcatacccgtacgacgttccggactacggttcccaccaccatcaccatcactag

SEQ ID NO: 7 - DNA, 423 bp, Homo sapiens
  source 1..423: mol_type = unassigned DNA
caggtgcagctgcaggagtctgggggaggattggtgcaggctgggggctctctgagactctcctgtgcagcctctggacgcaccttcagtaattataacatgggctggttccgccaggctccagggaaggagcgtgagtttgtagcagctattgactggagtggtggtagcccatactatgcagcctccgtgaggggccgattcaccatctccagagacaacgccgagaacacggtgtatctgcaaatgaacagcctgaaacctgaggacacggccgtttattactgtgcagctcctttatcgtacggcagtacctggttagctgactactggggccaggggacccaggtcaccgtctcctcagcggccgcatacccgtacgacgttccggactacggttcccaccaccatcaccatcactag

SEQ ID NO: 8 - DNA, 423 bp, Homo sapiens
  source 1..423: mol_type = unassigned DNA
caggtgcagctgcaggagtctggaggaggattggtgcaggctgggggctctctgagactctcctgtgcagcctctggacgcaccttcagtaactctaacatgggctggttccgccaggctccagggaaggagcgtgagtttgtagcagttattgactggagtggtggtagcccatactatacagactccgtgaggggccgattcaccatctccagagacaacgccaagaacacggtgtatctgcaaatgaacagactgaaacctgaggacacggccgtttattactgtgcaggaggcgtttccttcggtagtaggtggttgtccgactactggggccaggggacccaggtcaccgtctcctcagcggccgcatacccgtacgacgttccggactacggttcccaccaccatcaccatcactag

SEQ ID NO: 9 - DNA, 423 bp, Homo sapiens
  source 1..423: mol_type = unassigned DNA
caggtgcagctgcaggagtctgggggaggattggtgcaggctgggggctctctgagactctcctgtgcagcctctggacgcaccgtcggcagctattccatgggctggttccgccaggctccagggaaggagcgtgagtttgtagcagctgttatctggagtggtgctagtccatactatgcagactccgtgaagggccgattcaccatctccagagacaacgccaagaacacggtgtatctgcaaatgaacagcctgaaacctgaggacacggccgtttattactgtgcagcaaatcctacgtacagtggtggctggcacgcggaatactggggccaggggacccaggtcaccgtctcctcagcggccgcatacccgtacgacgttccggactacggttcccaccaccatcaccatcactag

SEQ ID NO: 10 - DNA, 423 bp, Homo sapiens
  source 1..423: mol_type = unassigned DNA
caggtgcagctgcaggagtctgggggaggattggtgcaggctgggggctctctgagactctcctgtgcagcctctggacgcaccgtcggcagctattccatgggctggttccgccaggctccagggaaggagcgtgagtttgtagcagctgttacctggagtggtgctagtccatactatgcagactccgtgaagggccgattcaccatctccagagacaacgccaagaacacggtgtatctgcaaatgaacagcctgaaacctgaggacacggccgtttattactgtgcagcaaatcctacgtacagtggtggctggcacgcggaatactggggccaggggacccaggtcaccgtctcctcagcggccgcatacccgtacgacgttccggactacggttcccaccaccatcaccatcactag

SEQ ID NO: 11 - DNA, 423 bp, Homo sapiens
  source 1..423: mol_type = unassigned DNA
caggtgcagctgcaggagtctgggggaggattggtgcaggctggggactctctgagactctcctgtgcagcctctggacgcaccgtcggcagctattccatgggctggttccgccaggctccagggaaggagcgtgagtttgtagcagctgttacctggagtggtgctagtccatactatgcagactccgtgaagggccgattcaccatctccagagacaacgccaagaacacggtgtatctgcaaatgaacagcctgaaacctgaggacacggccgtttattactgtgcagcaaatcctacgtacagtggtggctggcacgcggaatactggggccaggggacccaggtcaccgtctcctcagcggccgcatacccgtacgacgttccggactacggttcccaccaccatcaccatcactag

SEQ ID NO: 12 - DNA, 423 bp, Homo sapiens
  source 1..423: mol_type = unassigned DNA
caggtgcagctgcaggagtctgggggaggttcggagcagccggggggctctctgagactctcctgtgcagcctctggacgcaccgtcggcagctattccatgggctggttccgccaggctccagggaaggagcgtgagtttgtagcagctgttacccggagtggtgctagtccatactatgcagactccgtgaagggccgattcaccatctccagagacaacgccaagaacacggtgtatctgcaaatgaacagcctgaaacctgaggacacggccgtttattactgtgcagcaaatcctacgtacagtggtggctggcacgcggaatactggggccaggggacccaggtcaccgtctcctcagcggccgcatacccgtacgacgttccggactacggttcccaccaccatcaccatcactag

SEQ ID NO: 13 - DNA, 423 bp, Homo sapiens
  source 1..423: mol_type = unassigned DNA
caggtgcagctgcaggagtctgggggaggcttggtgcagcctggggggtctctgagactctcctgtgcagcctctagattcactttggattattatgccataggctggttccgccaggccccagggaaggagcgtgagtttgtagcagctgttacctggagtggtgctagtccatactatgcagactccgtgaagggccgattcaccatctccagagacaacgccaagaacacggtgtatctgcaaatgaacagcctgaaacctgaggacacggccgtttattactgtgcagcaaatcctacgtacagtggtggctggcacgcggaatactggggccaggggacccaggtcaccgtctcctcagcggccgcatacccgtacgacgttccggactacggttcccaccaccatcaccatcactag

SEQ ID NO: 14 - DNA, 423 bp, Homo sapiens
  source 1..423: mol_type = unassigned DNA
caggtgcagctgcaggagtctgggggaggcttggtgcaggctggggggtctctgagactctcctgtgcagcctctggacgctccttcagtagcgttaacatgggctggttccgccaggctccagggaaggagcgtgagttcgtagcggttattgactggagtggcggtagcccatactatacagactccgtgaggggccgattcaccatctccagagacaactccaagaacacggtgtatctgcaaatgaacagcctgaaacctgaggacacggccgtttattattgtgcagcaggggtttcgtacggtagtaggtggttgggggattactggggccaggggacccaggtcaccgtctcctcagcggccgcatacccgtacgacgttccggactacggttcccaccaccatcaccatcactag

SEQ ID NO: 15 - DNA, 414 bp, Homo sapiens
  source 1..414: mol_type = unassigned DNA
caggtgcagctgcaggagtctgggggaggattggcgcaggctgggggctctctgagactctcctgtgcagcctctggacgtaccttcagtatgggctggttccgccaggctccggggaaggagcgtgagtttgtagcagcaattacctatagtggtggtagtccgtactatgcgtcgtccgtgaggggccgattcaccatctccagagacaacgccaagaacacggtgtatctgcaaatgaacagcctgaaacctgaggacacggccgtttattactgcgcagcaaatcctacgtacggtagtgactggaacgcggaaaattggggccaggggacccaggtcaccgtctcctcagcggccgcatacccgtacgacgttccggactacggttcccaccaccatcaccatcactag

SEQ ID NO: 16 - DNA, 414 bp, Homo sapiens
  source 1..414: mol_type = unassigned DNA
caggtgcagctgcaggagtctggaggaggcttggtgcagcccgggggctctctgagactctcctgtgcagcctctggacgtaccttcagtatgggctggttccgccaggctccggggaaggagcgtgagtttgtagcagcaattacctatagtggtggtagtccgtactatgcgtcgtccgtgaggggccgattcaccatctccagagacaacgccaagaacacggtgtatctgcaaatgaacagcctgaaacctgaggacacggccgtttattactgcgcagcaaatcctacgtacggtagtgactggaacgcggaaaattggggccaggggacccaggtcaccgtctcctcagcggccgcatacccgtacgacgttccggactacggttcccaccaccatcaccatcactag

SEQ ID NO: 17 - DNA, 450 bp, Homo sapiens
  source 1..450: mol_type = unassigned DNA
caggtgcagctgcaggagtctgggggaggcttggtgcagcctggggggtctctgagactctcctgtacagcctctggattcactttggattattatgccataggctggctccgccaggccccagggaaggagcgtgagggggtctcatgtattagtagtagtggtggtagcacaaactatgcagactccgtgaagggccgattcaccatctccagagacaacgccaagaacacggtgtatctgctaatgaacagcctgaaacctgaggacacggccgtttattactgtgcagccgaacgaacatgggtcagtaattactactgttcaggcgacggagacggatatgactatgactactggggccaggggacccaggtcaccgtctcctcagcggccgcatacccgtacgacgttccggactacggttcccaccaccatcaccatcactag

SEQ ID NO: 18 - protein, 140 aa, Lama glama
QVQLQESGGGLVQAGGSLRLSCAASGRTFSRQSMGWFRQAPGKEREFVAVITWSGGSPYYADSVRGRFTISRDNAKNTVYLQMNSLKPEDTAVYYCAAPVSYGSQWLADYWGQGTQVTVSSAAAYPYDVPDYGSHHHHHH

SEQ ID NO: 19 - protein, 140 aa, Lama glama
QVQLQESGGGLVQAGDSLRLSCAASGRTFSRQSMGWFRQAPGKEREFVAVITWSGGSPYYADSVKGRFTISRDNAKNTVYLQMNSLKPEDTAVYYCAAPVSYGSQWLADYWGQGTQVTVSSAAAYPYDVPDYGSHHHHHH

SEQ ID NO: 20 - protein, 140 aa, Lama glama
QVQLQESGGGLVQAGGSLRLSCAASGRTFSGQSMGWFRQAPGKEREFVAVITWSGGSPYYADSVRGRFTISRDNAKNTVHLQMNSLKPEDTAVYYCAAPVSYGSQWLADYWGQGTQVTVSSAAAYPYDVPDYGSHHHHHH

SEQ ID NO: 21 - protein, 140 aa, Lama glama
QVQLQESGGGLVQAGGSLRLSCAASGRTFSSYAMGWFRQAPGKEREFVAVITWSGGSPYYADSVRGRFTISRDNAKNTVYLQMNSLKPEDTAVYYCAAPVSYGSQWLADYWGQGTQVTVSSAAAYPYDVPDYGSHHHHHH

SEQ ID NO: 22 - protein, 140 aa, Lama glama
QVQLQESGGGLVQAGGSLRLSCAASGRTFSRQSMGWFRQAPGEEREFVAVITWSGGSPYYADSVRGRFTISRDNAKNTVYLQMNSLKPEDTAVYYCAAPVSYGSQWLADYWGQGTQVTVSSAAAYPYDVPDYGSHHHHHH

SEQ ID NO: 23 - protein, 140 aa, Lama glama
QVQLQESGGGLVQAGGSLRLSCAASGRTFSSYNMGWFRQAPGKEREFVAVISWSGGSPYYADSVKGRFTISRDNAKNTVYLQMNSLKPEDTAVYYCAAPVSYGSSWLADYWGQGTQVTVSSAAAYPYDVPDYGSHHHHHH

SEQ ID NO: 24 - protein, 140 aa, Lama glama
QVQLQESGGGLVQAGGSLRLSCAASGRTFSNYNMGWFRQAPGKEREFVAAIDWSGGSPYYAASVRGRFTISRDNAENTVYLQMNSLKPEDTAVYYCAAPLSYGSTWLADYWGQGTQVTVSSAAAYPYDVPDYGSHHHHHH

SEQ ID NO: 25 - protein, 140 aa, Lama glama
QVQLQESGGGLVQAGGSLRLSCAASGRTFSNSNMGWFRQAPGKEREFVAVIDWSGGSPYYTDSVRGRFTISRDNAKNTVYLQMNRLKPEDTAVYYCAGGVSFGSRWLSDYWGQGTQVTVSSAAAYPYDVPDYGSHHHHHH

SEQ ID NO: 26 - protein, 140 aa, Lama glama
QVQLQESGGGLVQAGGSLRLSCAASGRSFSSVNMGWFRQAPGKEREFVAVIDWSGGSPYYTDSVRGRFTISRDNSKNTVYLQMNSLKPEDTAVYYCAAGVSYGSRWLGDYWGQGTQVTVSSAAAYPYDVPDYGSHHHHHH

SEQ ID NO: 27 - protein, 137 aa, Lama glama
QVQLQESGGGLAQAGGSLRLSCAASGRTFSMGWFRQAPGKEREFVAAITYSGGSPYYASSVRGRFTISRDNAKNTVYLQMNSLKPEDTAVYYCAANPTYGSDWNAENWGQGTQVTVSSAAAYPYDVPDYGSHHHHHH

SEQ ID NO: 28 - protein, 137 aa, Lama glama
QVQLQESGGGLVQPGGSLRLSCAASGRTFSMGWFRQAPGKEREFVAAITYSGGSPYYASSVRGRFTISRDNAKNTVYLQMNSLKPEDTAVYYCAANPTYGSDWNAENWGQGTQVTVSSAAAYPYDVPDYGSHHHHHH

SEQ ID NO: 29 - protein, 140 aa, Lama glama
QVQLQESGGGLVQAGGSLRLSCAASGRTVGSYSMGWFRQAPGKEREFVAAVIWSGASPYYADSVKGRFTISRDNAKNTVYLQMNSLKPEDTAVYYCAANPTYSGGWHAEYWGQGTQVTVSSAAAYPYDVPDYGSHHHHHH

SEQ ID NO: 30 - protein, 140 aa, Lama glama
QVQLQESGGGLVQAGGSLRLSCAASGRTVGSYSMGWFRQAPGKEREFVAAVTWSGASPYYADSVKGRFTISRDNAKNTVYLQMNSLKPEDTAVYYCAANPTYSGGWHAEYWGQGTQVTVSSAAAYPYDVPDYGSHHHHHH

SEQ ID NO: 31 - protein, 140 aa, Lama glama
QVQLQESGGGLVQAGDSLRLSCAASGRTVGSYSMGWFRQAPGKEREFVAAVTWSGASPYYADSVKGRFTISRDNAKNTVYLQMNSLKPEDTAVYYCAANPTYSGGWHAEYWGQGTQVTVSSAAAYPYDVPDYGSHHHHHH

SEQ ID NO: 32 - protein, 140 aa, Lama glama
QVQLQESGGGSEQPGGSLRLSCAASGRTVGSYSMGWFRQAPGKEREFVAAVTRSGASPYYADSVKGRFTISRDNAKNTVYLQMNSLKPEDTAVYYCAANPTYSGGWHAEYWGQGTQVTVSSAAAYPYDVPDYGSHHHHHH

SEQ ID NO: 33 - protein, 140 aa, Lama glama
QVQLQESGGGLVQPGGSLRLSCAASRFTLDYYAIGWFRQAPGKEREFVAAVTWSGASPYYADSVKGRFTISRDNAKNTVYLQMNSLKPEDTAVYYCAANPTYSGGWHAEYWGQGTQVTVSSAAAYPYDVPDYGSHHHHHH

SEQ ID NO: 34 - protein, 149 aa, Lama glama
QVQLQESGGGLVQPGGSLRLSCTASGFTLDYYAIGWLRQAPGKEREGVSCISSSGGSTNYADSVKGRFTISRDNAKNTVYLLMNSLKPEDTAVYYCAAERTWVSNYYCSGDGDGYDYDYWGQGTQVTVSSAAAYPYDVPDYGSHHHHHH

SEQ ID NO: 35 - protein, 10 aa, Lama glama
GRTFSRQSMG

SEQ ID NO: 36 - protein, 10 aa, Lama glama
GRTFSGQSMG

SEQ ID NO: 37 - protein, 10 aa, Lama glama
GRTFSSYAMG

SEQ ID NO: 38 - protein, 10 aa, Lama glama
GRTFSSYNMG

SEQ ID NO: 39 - protein, 10 aa, Lama glama
GRTFSNYNMG

SEQ ID NO: 40 - protein, 10 aa, Lama glama
GRTFSNSNMG

SEQ ID NO: 41 - protein, 10 aa, Lama glama
GRSFSSVNMG

SEQ ID NO: 42 - protein, 7 aa, Lama glama
GRTFSMG

SEQ ID NO: 43 - protein, 10 aa, Lama glama
GRTVGSYSMG

SEQ ID NO: 44 - protein, 10 aa, Lama glama
RFTLDYYAIG

SEQ ID NO: 45 - protein, 10 aa, Lama glama
GFTLDYYAIG

SEQ ID NO: 46 - protein, 17 aa, Lama glama
VITWSGGSPYYADSVRG

SEQ ID NO: 47 - protein, 17 aa, Lama glama
VITWSGGSPYYADSVKG

SEQ ID NO: 48 - protein, 17 aa, Lama glama
VISWSGGSPYYADSVKG

SEQ ID NO: 49 - protein, 17 aa, Lama glama
AIDWSGGSPYYAASVRG

SEQ ID NO: 50 - protein, 17 aa, Lama glama
VIDWSGGSPYYTDSVRG

SEQ ID NO: 51 - protein, 17 aa, Lama glama
AITYSGGSPYYASSVRG

SEQ ID NO: 52 - protein, 17 aa, Lama glama
AVIWSGASPYYADSVKG

SEQ ID NO: 53 - protein, 17 aa, Lama glama
AVTWSGASPYYADSVKG

SEQ ID NO: 54 - protein, 17 aa, Lama glama
AVTRSGASPYYADSVKG

SEQ ID NO: 55 - protein, 17 aa, Lama glama
CISSSGGSTNYADSVKG

SEQ ID NO: 56 - protein, 12 aa, Lama glama
PVSYGSQWLADY

SEQ ID NO: 57 - protein, 12 aa, Lama glama
PVSYGSSWLADY

SEQ ID NO: 58 - protein, 12 aa, Lama glama
PLSYGSTWLADY

SEQ ID NO: 59 - protein, 12 aa, Lama glama
GVSFGSRWLSDY

SEQ ID NO: 60 - protein, 12 aa, Lama glama
GVSYGSRWLGDY

SEQ ID NO: 61 - protein, 12 aa, Lama glama
NPTYGSDWNAEN

SEQ ID NO: 62 - protein, 12 aa, Lama glama
NPTYSGGWHAEY

SEQ ID NO: 63 - protein, 20 aa, Lama glama
ERTWVSNYYCSGDGDGYDYD

SEQ ID NO: 64 - DNA, 429 bp, Lama glama
  source 1..429: mol_type = unassigned DNA
caggtgcagctgcaggagtctgggggaggattggtgcaggctgggggctctctgagactctcctgtgcagcctctggacgcgacttcgctacctattccatggcctggttccgccaggctccagggaaggagcgtgagtctgtagcgacaattagctggagtggtcaacgtacacgctatgcggactccgtgaagggccgattcaccatctccagagacaacgccaagaacacggtgtatctgcaaatgaacagcctgaaacctgaggacacggccgtttattactgtgcaatgccccgtacctggggggagtttccacctacccagtatgactcgtggggccaggggacccaggtcaccgtctcctcagcggccgcatacccgtacgacgttccggactacggttcccaccaccatcaccatcactag

SEQ ID NO: 65 - DNA, 429 bp, Lama glama
  source 1..429: mol_type = unassigned DNA
caggtgcagctgcaggagtctgggggaggattggtgccggctgggggctctctgagactctcctgtgcagcctctggacgcgacttcgctacctattccatggcctggttccgccaggctccagggaaggagcgtgagtctgtagcgacaattagctggagtggtcaacgtacacgctatgcggactccgtgaagggccgattcaccatctccagagacaacgccaagaacacggtgtatctgcaaatgaacagcctgaaacctgaggacacggccgtttattactgtgcagcaccccgtacctggggggagtttccacctacccagtatgactcgtggggccaggggacccaggtcaccgtctcctcagcggccgcatacccgtacgacgttccggactacggttcccaccaccatcaccatcactag

SEQ ID NO: 66 - DNA, 429 bp, Lama glama
  source 1..429: mol_type = unassigned DNA
caggtgcagctgcaggagtctggaggaggattggtgcaggctgggggctctctgagactctcctgtgcagcctctggacgcgacttcgctacctattccatggcctggttccgccaggctccagggaaggagcgtgagtctgtagcgacaattagctggagtggtcaacgtacacgctatgcggactccgtgaagggccgattcaccatctccagagacaacgccaagaacacggtgtatctgcaaatgaacagcctgaaacctgaggacacggccgtttattactgtgcagcaccccgtacctggggggagtttccacctacccagtatgactcgtggggccaggggacccaggtcaccgtctcctcagcggccgcatacccgtacgacgttccggactacggttcccaccaccatcaccatcactag

SEQ ID NO: 67 - DNA, 429 bp, Lama glama
  source 1..429: mol_type = unassigned DNA
caggtgcagctgcaggagtctgggggaggattggtgcaggctgggggctctctgagactctcctgtgcagcctctggacgcgacttcgctacctattccatgacctggttccgccaggctccagggaaggagcgtgagtctgtagcgacaattagctggagtggtcaacgtacacgctatgcggactccgtgaagggccgattcaccatctccagagacaacgccaagaacacggtgtatctgcaaatgaacagcctgagacctgaggacacggccgtttattactgtgcagcaccccgtacctggggggagtttccacctacccagtatgactcgtggggccaggggacccaggtcaccgtctcctcagcggccgcatacccgtacgacgttccggactacggttcccaccaccatcaccatcactag

SEQ ID NO: 68 - DNA, 429 bp, Lama glama
  source 1..429: mol_type = unassigned DNA
caggtgcagctgcaggagtctgggggaggattggtgcaggctgggggctctctgagactctcctgtgcagcctctggacgcgacttcgctacctattccatggcctggttccgccaggctccaggggaggagcgtgagtctgtagcgacgattagctggagtggtcaacgtacacgctatgcggactccgtgaagggccgattcaccatctccagagacaacgccaagaacacggtgtatctgcaaatgaacagcctgaaacctgaggacacggccgtttattactgtgcagcaccccgtacctggggggagtttccacctacccagtatgactcgtggggccaggggacccaggtcaccgtctcctcagcggccgcatacccgtacgacgttccggactacggttcccaccaccatcaccatcactag

SEQ ID NO: 69 - DNA, 429 bp, Lama glama
  source 1..429: mol_type = unassigned DNA
caggtgcagctgcaggagtctgggggaggtttggtgcaggctggggactctctgagactctcctgcgcagcctctggacgcgacttcgctacctattccatggcctggttccgccaggctccagggaaggagcgtgagtctgtagcgacaattagctggagtggtcaacgtacacgctatgcggactccgtgaagggccgattcaccatctccagagacaacgccaagaacacggtgtatctgcaaatgaacagcctgaaacctgaggacacggccgtttattactgtgcagcaccccgtacctggggggagtttccacctacccagtatgactcgtggggccaggggacccaggtcaccgtctcctcagcggccgcatacccgtacgacgttccggactacggttcccaccaccatcaccatcactag

SEQ ID NO: 70 - DNA, 429 bp, Lama glama
  source 1..429: mol_type = unassigned DNA
caggtgcagctgcaggagtctggggggggcttggtgcagcctggggggtctctgagactctcctgtgcaacctctggacgcgacttcgctacctattccatggcctggttccgccaggctccagggaaggagcgtgagtctgtagcgacaattagctggagtggtcaacgtacacgctatgcggactccgtgaagggccgattcaccatctccagagacaacgccaagaacacggtgtatctgcaaatgaacagcctgaaacctgaggacacggccgtttattactgtgcagcaccccgtacctggggggagtttccacctacccagtatgactcgtggggccaggggacccaggtcaccgtctcctcagcggccgcatacccgtacgacgttccggactacggttcccaccaccatcaccatcactag

SEQ ID NO: 71 - DNA, 429 bp, Lama glama
  source 1..429: mol_type = unassigned DNA
caggtgcagctgcaggagtctgggggaggcttggtgcagcctggggggtctctgagactctcctgtgcagcctctggacgcgacttcgctacctattccatggcctggttccgccaggctccagggaaggagcgtgagtctgtagcgacaattagctggagtggtcaacgtacacgctatgcggactccgtgaagggccgattcaccatctccagagacaacgccaagaacacggtgtatctgcaaatgaacagcctgaaacctgaggacacggccgtttattactgtgcagcaccccgtacctggggggagtttccacctacccagtatgactcgtggggccaggggacccaggtcaccgtctcctcagcggccgcatacccgtacgacgttccggactacggttcccaccaccatcaccatcactag

SEQ ID NO: 72 - DNA, 429 bp, Lama glama
  source 1..429: mol_type = unassigned DNA
caggtgcagctgcaggagtctgggggaggcttggtgcaggctggggactctctgagactctcctgtgcagcctctggacgcgacttcagtacctattccatgggctggttccgccaggctccagggaaggagcgtgagtctgtagcgacaattagctggagtggtcaacgtacacgctatgcggactccgtgaaaggccgattcaccatctccagagacaacgccaagaacacggtgtatctgcaaatgaacagcctgaaacctgaggacacggccgtttattactgtgcagcaccccgtacctggggggagtttccacctacccagtatgactcgtggggccaggggacccaggtcaccgtctcctcagcggccgcatacccgtacgacgttccggactacggttcccaccaccatcaccatcactag

SEQ ID NO: 73 - DNA, 429 bp, Lama glama
  source 1..429: mol_type = unassigned DNA
caggtgcagctgcaggagtctgggggaggctcggtgcagactgggggctctctgagactctcctgtgcagcctctggacgcgacttcagtacctattccatgggctggttccgccaggctccagggaaggagcgtgagtctgtagcgacaattagctggagtggtcaacgtacacgctatgcggactccgtgaagggccgattcaccatctccagagacaacgccaagaacacggtgtatctgcaaatgaacagcctgaaacctgaggacacggccgtttattactgtgcagcaccccgtacctggggggagtttccacctacccagtatgactcgtggggccaggggacccaggtcaccgtctcctcagcggccgcatacccgtacgacgttccggactacggttcccaccaccatcaccatcactag

SEQ ID NO: 74 - DNA, 429 bp, Lama glama
  source 1..429: mol_type = unassigned DNA
caggtgcagctgcaggagtctggaggaggattggtgcaggctgggggctctctgagactctcctgtgcagcctctggacgcaccttcagtacatattccatgggctggttccgccaggctccagggaaggagcgtgagtttgtagcgattattagctggagtggtcaacgtacacgctatgcggactccgtgaagggccgattcaccatctccagagacaacgccaagaacacggtgtatctgcaaatgaacagcctgaaacctgaggacacggccgtttattactgtgcagcaccccgtacctggggggagtttccacctacccagtatgactcgtggggccaggggacccaggtcaccgtctcctcagcggccgcatacccgtacgacgttccggactacggttcccaccaccatcaccatcactag

SEQ ID NO: 75 - DNA, 429 bp, Lama glama
  source 1..429: mol_type = unassigned DNA
caggtgcagctgcaggagtctgggggaggattggtgcaggctgggggctctctgagactctcctgtgtagcctctggacgcaccttcaatacctattccatgggctggttccgccaggctccagggaaggagcgtgagtttgtagcgtctattagctggagtggtcaacgttcacgctatgcggactccgtgaagggccgattcaccatctccagagacaacgccaagaacacggtgtatctgcaaatgaacagcctgaaacctgaggacacggccgtttattactgtgcgtcaccccgtacctggggggagtttccacctactcagtatgactcgtggggccaggggacccaggtcaccgtctcctcagcggccgcatacccgtacgacgttccggactacggttcccaccaccatcaccatcactag

SEQ ID NO: 76 - DNA, 426 bp, Lama glama
  source 1..426: mol_type = unassigned DNA
caggtgcagctgcaggagtctgggggaggattggtgcaggctgagggctctctgagactctcgtgtgcagcctctggacgcacccgtgatgccaatgccatgggctggttccgccaggctccagggaaggagcgtgagttagtagcagctattagctggagtggtagtaggacatactatgcagactccgtgaagggccgattcaccatctccagagacaatgtcatgcacacggtgtatctgtcaatgaatagcctgaaacctgaggacacggccgtttattattgtgcagctgatcgaagcattgaggtccaaatcgcggattatgactactggggccgggggacccaggtcaccgtctcctcagcggccgcatacccgtacgacgttccggactacggttcccaccaccatcaccatcactag

SEQ ID NO: 77 - DNA, 426 bp, Lama glama
  source 1..426: mol_type = unassigned DNA
caggtgcagctgcaggagtctgggggaggattggcgcaggctgggaactctctgagaatctcttgtgtagcctctggaaacaccttcgacacacgtgccatgggctggttccgccaggctccagggaaggagcgtgagtttgtagcggcgattagtcggagtagtttcaacacatactactccgactccgtgacgggccgattcaccatctccagagacaacgccaagaacacggtgtatctgcaaatgaacagcctgaaacctgaggacacggccgtttattactgtgtagctggcaagtacggtatgaagtggagggatggcgctgactactggggccaggggacccaggtcaccgtctcctcagcggccgcatacccgtacgacgttccggactacggttcccaccaccatcaccatcactag

SEQ ID NO: 78 - DNA, 426 bp, Lama glama
  source 1..426: mol_type = unassigned DNA
caggtgcagctgcaggagtctgggggaggattggcgcaggctgggaactctctgagaatctcttgtgtagcctctggaaacaccttcgacacacgtgccatgggctggttccgccaggctccagggaaggagcgtgagtttgtagcggcgattagtcggagtagtttcaacacatactactccgactccgtgacgggccgattcaccatctccagagacaacgccaagaacacggtgtatctgcaaatgaacagcctgaaacctgaggacacggccgtttattactgtgcagctggcaagtacggtatgaagtggagggatggcgctgactactggggccaggggacccaggtcaccgtctcctcagcggccgcatacccgtacgacgttccggactacggttcccaccaccatcaccatcactag

SEQ ID NO: 79 - DNA, 426 bp, Lama glama
  source 1..426: mol_type = unassigned DNA
caggtgcagctgcaggagtctgggggaggcttggcgcaggagggggggtccctgagactctcttgtgtagcctctggaaacaccttcgacacacgtgccatgggctggttccgccaggctccagggaaggagcgtgagtttgtagcggcgattagtcggagtagtttcaacacatactactccgactccgtgacgggccgattcaccatctccagagacaacgccaagaacatggtgtatctgcaaatgaacagcctgaaacctgaggacacggccgtttattactgtgcagctggcaagtacggtatgaagtggagggatggcgctgactactggggccaggggacccaggtcaccgtctcctcagcggccgcatacccgtacgacgttccggactacggttcccaccaccatcaccatcactag

SEQ ID NO: 80 - DNA, 426 bp, Lama glama
  source 1..426: mol_type = unassigned DNA
caggtgcagctgcaggagtctggaggaggcttggtgcaggctggggagtctctgagaatctcttgtgtagcctctggaaacaccttcgacacacgtgccatgggctggttccgccaggctccagggaaggagcgtgagtttgtagcggcgattagtcggagtagtttcaacacatactactccgactccgtgacgggccgattcaccatctccagagacaacgccaagaacacggtgtatctgcaaatgaacagcctgaaacctgaggacacggccgtttattactgtgtagctggcaagtacggtatgaagtggagggatggcgctgactactggggccaggggacccaggtcaccgtctcctcagcggccgcatacccgtacgacgttccggactacggttcccaccaccatcaccatcactag

SEQ ID NO: 81 - DNA, 426 bp, Lama glama
  source 1..426: mol_type = unassigned DNA
caggtgcagctgcaggagtctgggggaggattggtgcagactgggggctctctgagactctcctgtgcagcctctggaaacaccttcgacacacgtgccatgggctggttccgccaggctccagggaaggagcgtgagtttgtagcggcgattagtcggagtagtttcaacacatactactccgactccgtgacgggccgattcaccatctccagagacaacgccaagaacacggtgtatctgcaaatgaacagcctgaaacctgaggacacggccgtttattactgtgcagctggcaagtacggtatgaagtggagggatggcgctgactactggggccaggggacccaggtcaccgtctcctcagcggccgcatacccgtacgacgttccggactacggttcccaccaccatcaccatcactag

SEQ ID NO: 82 - DNA, 426 bp, Lama glama
  source 1..426: mol_type = unassigned DNA
caggtgcagctgcaggagtctgggggaggatcggtacagactgggggcactctgacactctcttgtgtagcctctggaaacaccttcgacacacgtgccatgggctggttccgccaggctccaggggaggagcgtgagtttgtagcggcgattagtcggagtagtttcaacacatactactccgactccgtgacgggccgattcaccatctccagagacaacgccaagaacacggtgtatctgcaaatgaacagcctgaaacctgaggacacggccgtttattactgtgcagctggcaagtacggtatgaagtggagggatggcgctgactactggggccaggggacccaggtcaccgtctcctcagcggccgcatacccgtacgacgttccggactacggttcccaccaccatcaccatcactag

SEQ ID NO: 83 - DNA, 423 bp, Lama glama
  source 1..423: mol_type = unassigned DNA
caggtgcagctgcaggagtctgggggaggatcggtgcaggctgggggttctctgagactctcctgtgcagcctccggaagcaccttcagtatcaaggccatggggtggtaccgccaggctccagggaagcagcgcgagttggtcgcagcttttattagtggtcgtggtagtacaaagtatgcagactccgtgaagggccgattcgccatctccagagacaatgccaagaacacgatgtatctgcaaatggacagcctggaacctgaggacacggccgtgtattactgttacatagtactgcctactggggggggaagcgccatggactactggggcgaagggacccaggtcaccgtctcctcagcggccgcatacccgtacgacgttccggactacggttcccaccaccatcaccatcactag

SEQ ID NO: 84 - DNA, 423 bp, Lama glama
  source 1..423: mol_type = unassigned DNA
caggtgcagctgcaggagtctgggggaggcgtcgtgcaggctgggggttctctgagactctcctgtgcagcctccggaagcaccttcagtatcaaggccatggggtggtaccgccaggctccagggaagcagcgcgacttggtcgcaggtttcattagtggtcgtggtagtgcaaagtatgcagactccgtgaagggccgattcgccatctccagagacaatgccaagaacacgatgtatctgcaaatggacagcctgaaacctgaggacacggccgtgtattactgctacatagtactgactactggggggggaagcgccatggactactggggccaagggacccaggtcaccgtctcctcagcggccgcatacccgtacgacgttccggactacggttcccaccaccatcaccatcactag

SEQ ID NO: 85 - protein, 142 aa, Lama glama
QVQLQESGGGLVQAGGSLRLSCAASGRDFATYSMAWFRQAPGKERESVATISWSGQRTRYADSVKGRFTISRDNAKNTVYLQMNSLKPEDTAVYYCAMPRTWGEFPPTQYDSWGQGTQVTVSSAAAYPYDVPDYGSHHHHHH

SEQ ID NO: 86 - protein, 142 aa, Lama glama
QVQLQESGGGLVQAGGSLRLSCAASGRDFATYSMAWFRQAPGKERESVATISWSGQRTRYADSVKGRFTISRDNAKNTVYLQMNSLKPEDTAVYYCAAPRTWGEFPPTQYDSWGQGTQVTVSSAAAYPYDVPDYGSHHHHHH

SEQ ID NO: 87 - protein, 142 aa, Lama glama
QVQLQESGGGLVPAGGSLRLSCAASGRDFATYSMAWFRQAPGKERESVATISWSGQRTRYADSVKGRFTISRDNAKNTVYLQMNSLKPEDTAVYYCAAPRTWGEFPPTQYDSWGQGTQVTVSSAAAYPYDVPDYGSHHHHHH

SEQ ID NO: 88 - protein, 142 aa, Lama glama
QVQLQESGGGLVQAGDSLRLSCAASGRDFATYSMAWFRQAPGKERESVATISWSGQRTRYADSVKGRFTISRDNAKNTVYLQMNSLKPEDTAVYYCAAPRTWGEFPPTQYDSWGQGTQVTVSSAAAYPYDVPDYGSHHHHHH

SEQ ID NO: 89 - protein, 142 aa, Lama glama
QVQLQESGGGLVQAGGSLRLSCAASGRDFATYSMAWFRQAPGEERESVATISWSGQRTRYADSVKGRFTISRDNAKNTVYLQMNSLKPEDTAVYYCAAPRTWGEFPPTQYDSWGQGTQVTVSSAAAYPYDVPDYGSHHHHHH

SEQ ID NO: 90 - protein, 142 aa, Lama glama
QVQLQESGGGLVQPGGSLRLSCAASGRDFATYSMAWFRQAPGKERESVATISWSGQRTRYADSVKGRFTISRDNAKNTVYLQMNSLKPEDTAVYYCAAPRTWGEFPPTQYDSWGQGTQVTVSSAAAYPYDVPDYGSHHHHHH

SEQ ID NO: 91 - protein, 142 aa, Lama glama
QVQLQESGGGLVQPGGSLRLSCATSGRDFATYSMAWFRQAPGKERESVATISWSGQRTRYADSVKGRFTISRDNAKNTVYLQMNSLKPEDTAVYYCAAPRTWGEFPPTQYDSWGQGTQVTVSSAAAYPYDVPDYGSHHHHHH

SEQ ID NO: 92 - protein, 142 aa, Lama glama
QVQLQESGGGLVQAGGSLRLSCAASGRDFATYSMTWFRQAPGKERESVATISWSGQRTRYADSVKGRFTISRDNAKNTVYLQMNSLRPEDTAVYYCAAPRTWGEFPPTQYDSWGQGTQVTVSSAAAYPYDVPDYGSHHHHHH

SEQ ID NO: 93 - protein, 142 aa, Lama glama
QVQLQESGGGLVQAGDSLRLSCAASGRDFSTYSMGWFRQAPGKERESVATISWSGQRTRYADSVKGRFTISRDNAKNTVYLQMNSLKPEDTAVYYCAAPRTWGEFPPTQYDSWGQGTQVTVSSAAAYPYDVPDYGSHHHHHH

SEQ ID NO: 94 - protein, 142 aa, Lama glama
QVQLQESGGGLVQAGGSLRLSCVASGRTFNTYSMGWFRQAPGKEREFVASISWSGQRSRYADSVKGRFTISRDNAKNTVYLQMNSLKPEDTAVYYCASPRTWGEFPPTQYDSWGQGTQVTVSSAAAYPYDVPDYGSHHHHHH

SEQ ID NO: 95 - protein, 142 aa, Lama glama
QVQLQESGGGLVQAGGSLRLSCAASGRTFSTYSMGWFRQAPGKEREFVAIISWSGQRTRYADSVKGRFTISRDNAKNTVYLQMNSLKPEDTAVYYCAAPRTWGEFPPTQYDSWGQGTQVTVSSAAAYPYDVPDYGSHHHHHH

SEQ ID NO: 96 - protein, 142 aa, Lama glama
QVQLQESGGGSVQTGGSLRLSCAASGRDFSTYSMGWFRQAPGKERESVATISWSGQRTRYADSVKGRFTISRDNAKNTVYLQMNSLKPEDTAVYYCAAPRTWGEFPPTQYDSWGQGTQVTVSSAAAYPYDVPDYGSHHHHHH

SEQ ID NO: 97 - protein, 141 aa, Lama glama
QVQLQESGGGLAQAGNSLRISCVASGNTFDTRAMGWFRQAPGKEREFVAAISRSSFNTYYSDSVTGRFTISRDNAKNTVYLQMNSLKPEDTAVYYCAAGKYGMKWRDGADYWGQGTQVTVSSAAAYPYDVPDYGSHHHHHH

SEQ ID NO: 98 - protein, 141 aa, Lama glama
QVQLQESGGGLAQAGNSLRISCVASGNTFDTRAMGWFRQAPGKEREFVAAISRSSFNTYYSDSVTGRFTISRDNAKNTVYLQMNSLKPEDTAVYYCVAGKYGMKWRDGADYWGQGTQVTVSSAAAYPYDVPDYGSHHHHHH

SEQ ID NO: 99 - protein, 141 aa, Lama glama
QVQLQESGGGLVQAGESLRISCVASGNTFDTRAMGWFRQAPGKEREFVAAISRSSFNTYYSDSVTGRFTISRDNAKNTVYLQMNSLKPEDTAVYYCVAGKYGMKWRDGADYWGQGTQVTVSSAAAYPYDVPDYGSHHHHHH

SEQ ID NO: 100 - protein, 141 aa, Lama glama
QVQLQESGGGLAQEGGSLRLSCVASGNTFDTRAMGWFRQAPGKEREFVAAISRSSFNTYYSDSVTGRFTISRDNAKNMVYLQMNSLKPEDTAVYYCAAGKYGMKWRDGADYWGQGTQVTVSSAAAYPYDVPDYGSHHHHHH

SEQ ID NO: 101 - protein, 141 aa, Lama glama
QVQLQESGGGLVQTGGSLRLSCAASGNTFDTRAMGWFRQAPGKEREFVAAISRSSFNTYYSDSVTGRFTISRDNAKNTVYLQMNSLKPEDTAVYYCAAGKYGMKWRDGADYWGQGTQVTVSSAAAYPYDVPDYGSHHHHHH

SEQ ID NO: 102 - protein, 141 aa, Lama glama
QVQLQESGGGSVQTGGTLTLSCVASGNTFDTRAMGWFRQAPGEEREFVAAISRSSFNTYYSDSVTGRFTISRDNAKNTVYLQMNSLKPEDTAVYYCAAGKYGMKWRDGADYWGQGTQVTVSSAAAYPYDVPDYGSHHHHHH

SEQ ID NO: 103 - protein, 141 aa, Lama glama
QVQLQESGGGLVQAEGSLRLSCAASGRTRDANAMGWFRQAPGKERELVAAISWSGSRTYYADSVKGRFTISRDNVMHTVYLSMNSLKPEDTAVYYCAADRSIEVQIADYDYWGRGTQVTVSSAAAYPYDVPDYGSHHHHHH

SEQ ID NO: 104 - protein, 140 aa, Lama glama
QVQLQESGGGSVQAGGSLRLSCAASGSTFSIKAMGWYRQAPGKQRELVAAFISGRGSTKYADSVKGRFAISRDNAKNTMYLQMDSLEPEDTAVYYCYIVLPTGGGSAMDYWGEGTQVTVSSAAAYPYDVPDYGSHHHHHH

SEQ ID NO: 105 - protein, 140 aa, Lama glama
QVQLQESGGGVVQAGGSLRLSCAASGSTFSIKAMGWYRQAPGKQRDLVAGFISGRGSAKYADSVKGRFAISRDNAKNTMYLQMDSLKPEDTAVYYCYIVLTTGGGSAMDYWGQGTQVTVSSAAAYPYDVPDYGSHHHHHH

SEQ ID NO: 106 - protein, 10 aa, Lama glama
GRDFATYSMA

SEQ ID NO: 107 - protein, 10 aa, Lama glama
GRDFATYSMT

SEQ ID NO: 108 - protein, 10 aa, Lama glama
GRDFSTYSMG

SEQ ID NO: 109 - protein, 10 aa, Lama glama
GRTFNTYSMG

SEQ ID NO: 110 - protein, 10 aa, Lama glama
GRTFSTYSMG

SEQ ID NO: 111 - protein, 10 aa, Lama glama
GRDFSTYSMG

SEQ ID NO: 112 - protein, 10 aa, Lama glama
GNTFDTRAMG

SEQ ID NO: 113 - protein, 10 aa, Lama glama
GRTRDANAMG

SEQ ID NO: 114 - protein, 10 aa, Lama glama
GSTFSIKAMG

SEQ ID NO: 115 - protein, 17 aa, Lama glama
TISWSGQRTRYADSVKG

SEQ ID NO: 116 - protein, 17 aa, Lama glama
SISWSGQRSRYADSVKG

SEQ ID NO: 117 - protein, 17 aa, Lama glama
IISWSGQRTRYADSVKG

SEQ ID NO: 118 - protein, 17 aa, Lama glama
AISRSSFNTYYSDSVTG

SEQ ID NO: 119 - protein, 17 aa, Lama glama
AISWSGSRTYYADSVKG

SEQ ID NO: 120 - protein, 17 aa, Lama glama
AFISGRGSTKYADSVKG

SEQ ID NO: 121 - protein, 17 aa, Lama glama
GFISGRGSAKYADSVKG

SEQ ID NO: 122 - protein, 14 aa, Lama glama
PRTWGEFPPTQYDS

SEQ ID NO: 123 - protein, 13 aa, Lama glama
GKYGMKWRDGADY

SEQ ID NO: 124 - protein, 13 aa, Lama glama
DRSIEVQIADYDY

SEQ ID NO: 125 - protein, 12 aa, Lama glama
VLPTGGGSAMDY

SEQ ID NO: 126 - protein, 12 aa, Lama glama
VLTTGGGSAMDY

SEQ ID NO: 127 - protein, 165 aa, synthetic construct
  REGION 1..165: note = IFN-alpha2a
CDLPQTHSLGSRRTLMLLAQMRKISLFSCLKDRHDFGFPQEEFGNQFQKAETIPVLHEMIQQIFNLFSTKDSSAAWDETLLDKFYTELYQQLNDLEACVIQGVGVTETPLMKEDSILAVRKYFQRITLYLKEKKYSPCAWEVVRAEIMRSFSLSTNLQESLRSKE

SEQ ID NO: 128 - protein, 165 aa, synthetic construct [sequence omitted]

SEQ ID NO: 129 - protein, 297 aa, Homo sapiens
MTTPRNSVNGTFPAEPMKGPIAMQSGPKPLFRRMSSLVGPTQSFFMRESKTLGAVQIMNGLFHIALGGLLMIPAGIYAPICVTVWYPLWGGIMYIISGSLLAATEKNSRKCLVKGKMIMNSLSLFAAISGMILSIMDILNIKISHFLKMESLNFIRAHTPYINIYNCEPANPSEKNSPSTQYCYSIQSLFLGILSVMLIFAFFQELVIAGIVENEWKRTCSRPKSNIVLLSAEEKKEQTIEIKEEVVGLTETSSQPKNEEDIEIIPIQEEEEEETETNFPEPPQDQESSPIENDSSP

SEQ ID NO: 130 - protein, 157 aa, Homo sapiens [sequence omitted]

SEQ ID NO: 131 - protein, 171 aa, Homo sapiens
LPGVGLTPSAAQTARQHPKMHLAHSNLKPAAHLIGDPSKQNSLLWRANTDRAFLQDGFSLSNNSLLVPTSGIYFVYSQVVFSGKAYSPKATSSPLYLAHEVQLFSSQYPFHVPLLSSQKMVYPGLQEPWLHSMYHGAAFQLTQGDQLSTHTDGIPHLVLSPSTVFFGAFAL

SEQ ID NO: 132 - protein, 281 aa, Homo sapiens [sequence omitted]

SEQ ID NO: 133 - protein, 153 aa, Homo sapiens
APVRSLNCTLRDSQQKSLVMSGPYELKALHLQGQDMEQQVVFSMSFVQGEESNDKIPVALGLKEKNLYLSCVLKDDKPTLQLESVDPKNYPKKKMEKRFVFNKIEINNKLEFESAQFPNWYISTSQAENMPVFLGGTKGGQDITDFTMQFVSS

SEQ ID NO: 134 - protein, 133 aa, Homo sapiens [sequence omitted]

SEQ ID NO: 135 - protein, 129 aa, Homo sapiens [sequence omitted]

SEQ ID NO: 136 - protein, 185 aa, Homo sapiens
APVPPGEDSKDVAAPHRQPLTSSERIDKQIRYILDGISALRKETCNKSNMCESSKEALAENNLNLPKMAEKDGCFQSGFNEETCLVKIITGLLEFEVYLEYLQNRFESSEEQARAVQMSTKVLIQFLQKKAKNLDAITTPDPTTNASLTTKLQAQNQWLQDMTTHLILRSFKEFLQSSLRALRQM

SEQ ID NO: 137 - protein, 114 aa, Homo sapiens
SPGPVPPSTALRELIEELVNITQNQKAPLCNGSMVWSINLTAGMYCAALESLINVSGCSAIEKTQRMLSGFCPHKVSAGQFSSLHVRDTKIEVAQFVKDLLLHLKKLFREGRFN

SEQ ID NO: 138 - protein, 194 aa, Homo sapiens
MAAEPVEDNCINFVAMKFIDNTLYFIAEDDENLESDYFGKLESKLSVIRNLNDQVLFIDQGNRPLFEDMTDSDCRDNAPRTIFIISMYKDSQPRGMAVTISVKCEKISTLSCENKIISFKEMNPPDNIKDTKSDIIFFQRSVPGHDNKMQFESSSYEGYFLACEKERDLFKLILKKEDELGDRSIMFTVQNEDL

SEQ ID NO: 139 - protein, 270 aa, Homo sapiens
MKPKMKYSTNKISTAKWKNTASKALCFKLGKSQQKAKEVCPMYFMKLRSGLMIKKEACYFRRETTKRPSLKTGRKHKRHLVLAACQQQSTVECFAFGISGVQKYTRALHDSSITGISPITEYLASLSTYNDQSITFALEDESYEIYVEDLKKDEKKDKVLLSYYESQHPSNESGDGVDGKMLMVTLSPTKDFWLHANNKEHSVELHKCEKPLPDQAFFVLHNMHSNCVSFECKTDPGVFIGVKDNHLALIKVDSSENLCTENILFKLSET

SEQ ID NO: 140 - protein, 119 aa, Homo sapiens
EVQLVESGGGLVQAGKSLRLSCAASGSIFSIHAMGWFRQAPGKEREFVAAITWSGGITYYEDSVKGRFTISRDNAKNTVYLQMNSLKPEDTAIYYCAADRAESSWYDYWGQGTQVTVSS

SEQ ID NO: 141 - protein, 123 aa, Homo sapiens
EVQLVESGGGLVQPGGSLRLSCAASGFTLDYYAKCWFRQAPGKEREWVSCISSSDGSTYYADSVKGRFTISRDNAKNTVYLQMNSLKPEDTAVYFCAARHGGPLTVEYFFDYWGQGTQVTVSS

SEQ ID NO: 142 - protein, 16 aa, synthetic construct
  REGION 1..16: note = Linker
GGSGGSGGGGSGGGGS

SEQ ID NO: 143 - DNA, 40 bp, synthetic construct
  misc_feature 1..40: note = primer
  source 1..40: mol_type = other DNA
gataagatctcaggcggatccacaacacccagaaattcag

SEQ ID NO: 144 - DNA, 42 bp, synthetic construct
  misc_feature 1..42: note = primer
  source 1..42: mol_type = other DNA
ggttttttctctagatcaaggagagctgtcattttctattgg

SEQ ID NO: 145 - DNA, 20 bp, synthetic construct
  misc_feature 1..20: note = primer
  source 1..20: mol_type = other DNA
ttatgcttccggctcgtatg

SEQ ID NO: 146 - DNA, 29 bp, synthetic construct
  misc_feature 1..29: note = primer
  misc_feature 24: note = r can be a or g
  source 1..29: mol_type = other DNA
gatgtgcagctgcaggagtctggrggagg

SEQ ID NO: 147 - DNA, 34 bp, synthetic construct
  misc_feature 1..34: note = primer
  source 1..34: mol_type = other DNA
ctagtgcggccgctgaggagacggtgacctgggt

SEQ ID NO: 148 - DNA, 22 bp, synthetic construct
  misc_feature 1..22: note = primer
  source 1..22: mol_type = other DNA
tcacacaggaaacagctatgac

SEQ ID NO: 149 - DNA, 24 bp, synthetic construct
  misc_feature 1..24: note = primer
  source 1..24: mol_type = other DNA
cgccagggttttcccagtcacgac

SEQ ID NO: 150 - DNA, 43 bp, synthetic construct
  misc_feature 1..43: note = primer
  source 1..43: mol_type = other DNA
gataagatctcaggcggatccagtggacctttcccagcagagc

SEQ ID NO: 151 - DNA, 41 bp, synthetic construct
  misc_feature 1..41: note = primer
  source 1..41: mol_type = other DNA
ggttttttctctagatcaaggagcgatctcattttccactg

SEQ ID NO: 152 - protein, 5 aa, synthetic construct
  REGION 1..5: note = Linker
GGGGS

SEQ ID NO: 153 - protein, 10 aa, synthetic construct
  REGION 1..10: note = Linker
GGGGSGGGGS

SEQ ID NO: 154 - protein, 15 aa, synthetic construct
  REGION 1..15: note = linker
GGGGSGGGGSGGGGS

SEQ ID NO: 155 - protein, 20 aa, synthetic construct
  REGION 1..20: note = linker
GGGGSGGGGSGGGGSGGGGS

SEQ ID NO: 156 - protein, 8 aa, synthetic construct
  REGION 1..8: note = linker
GGGGGGGG

SEQ ID NO: 157 - protein, 6 aa, synthetic construct
  REGION 1..6: note = linker
GGGGGG

SEQ ID NO: 158 - protein, 5 aa, synthetic construct
  REGION 1..5: note = linker
EAAAK

SEQ ID NO: 159 - protein, 10 aa, synthetic construct
  REGION 1..10: note = linker
EAAAKEAAAK

SEQ ID NO: 160 - protein, 15 aa, synthetic construct
  REGION 1..15: note = linker
EAAAKEAAAKEAAAK

SEQ ID NO: 161 - protein, 12 aa, synthetic construct
  REGION 1..12: note = linker
AEAAAKEAAAKA

SEQ ID NO: 162 - protein, 17 aa, synthetic construct
  REGION 1..17: note = linker
AEAAAKEAAAKEAAAKA

SEQ ID NO: 163 - protein, 22 aa, synthetic construct
  REGION 1..22: note = linker
AEAAAKEAAAKEAAAKEAAAKA

SEQ ID NO: 164 - protein, 27 aa, synthetic construct
  REGION 1..27: note = linker
AEAAAKEAAAKEAAAKEAAAKEAAAKA

SEQ ID NO: 165 - protein, 46 aa, synthetic construct
  REGION 1..46: note = linker
AEAAAKEAAAKEAAAKEAAAKALEAEAAAKEAAAKEAAAKEAAAKA

SEQ ID NO: 166 - protein, 5 aa, synthetic construct
  REGION 1..5: note = linker
PAPAP

SEQ ID NO: 167 - protein, 18 aa, synthetic construct
  REGION 1..18: note = linker
KESGSVSSEQLAQFRSLD

SEQ ID NO: 168 - protein, 14 aa, synthetic construct
  REGION 1..14: note = linker
EGKSSGSGSESKST

SEQ ID NO: 169 - protein, 12 aa, synthetic construct
  REGION 1..12: note = linker
GSAGSAAGSGEF